European Patent Specification EP 3 373 968 B1, published April 17, 2024. Title: GLYPICAN 2 AS A CANCER MARKER AND THERAPEUTIC TARGET. Applicant: The Children's Hospital of Philadelphia The Government of the United States of America as represented by the Secretary of the Department of Health and Human Services. Application Unknown. The sequence listing filed with the application follows.

SEQUENCE LISTING (30 sequences)

SEQ ID NO: 1 - DNA, 357 bp, Artificial sequence
  Synthetic oligonucleotide
gaggtgcagctggtggagactgggggaggcgtggtcaagcctggagggtccctgagactctcctgtgcagcctctggattcaccttcagtgactactacatgagctggatccgccaggctccagggaaggggctggagtgggtttcatacattagtagtagtggtagtaccatatactacgcagactccgtgaagggccgattcaccatctccagagacaattccaagaacacgctgtatctgcaaatgaacagcctgagagctgaggacacggctgtgtattactgtgcgagagagagtggctacgattacgtgtttgactactggggccagggaaccctggtcgccgtctcctca

SEQ ID NO: 2 - protein, 119 aa, Artificial sequence
  Synthetic amino acid
EVQLVETGGGVVKPGGSLRLSCAASGFTFSDYYMSWIRQAPGKGLEWVSYISSSGSTIYYADSVKGRFTISRDNSKNTLYLQMNSLRAEDTAVYYCARESGYDYVFDYWGQGTLVAVSS

SEQ ID NO: 3 - DNA, 324 bp, Artificial sequence
  Synthetic oligonucleotide
gacatccagatgacccagtctccttccaccctgtctgcatttgtaggagacagagtcaccatcacttgccgggccagtcagagtattagtagctggttggcctggtatcagcaaaaaccagggaaagcccctaagctcctgatctatgctgcatccactttgcaaagtggggtcccatcaaggttcagcggcagtggatctgggacagaattcactctcacaatcagcagcctgcagcctgaagattttgcaacttattactgtcaacagcttaatagttaccctatcaccttcggccaagggacacgactggagattaaacga

SEQ ID NO: 4 - protein, 108 aa, Artificial sequence
  Synthetic amino acid
DIQMTQSPSTLSAFVGDRVTITCRASQSISSWLAWYQQKPGKAPKLLIYAASTLQSGVPSRFSGSGSGTEFTLTISSLQPEDFATYYCQQLNSYPITFGQGTRLEIKR

SEQ ID NO: 5 - protein, 8 aa, Artificial sequence
  Synthetic amino acid
GFTFSDYY

SEQ ID NO: 6 - protein, 8 aa, Artificial sequence
  Synthetic amino acid
ISSSGSTI

SEQ ID NO: 7 - protein, 12 aa, Artificial sequence
  Synthetic amino acid
ARESGYDYVFDY

SEQ ID NO: 8 - protein, 6 aa, Artificial sequence
  Synthetic amino acid
QSISSW

SEQ ID NO: 9 - protein, 3 aa, Artificial sequence
  Synthetic amino acid
AAS

SEQ ID NO: 10 - protein, 9 aa, Artificial sequence
  Synthetic amino acid
QQLNSYPIT

SEQ ID NO: 11 - DNA, 345 bp, Artificial sequence
  Synthetic oligonucleotide
caggtgcagctggtgcagtctggaggaggcttgatccagcctggggggtccctgagactctcctgtgcagcctctgggttcaccgtcagtagcaactacatgagctgggtccgccaggctccagggaaggggctggagtgggtctcagttatttatagcggtggtagcacatactacgcagactccgtgaagggccgattcaccatctccagagacaattccaagaacacgctgtatcttcaaatgaacagcctgagagccgaggacacggccgtgtattactgtgcgagagattcgaatgcttttgatatctggggccaagggacaatggtcaccgtctcttca

SEQ ID NO: 12 - protein, 115 aa, Artificial sequence
  Synthetic amino acid
QVQLVQSGGGLIQPGGSLRLSCAASGFTVSSNYMSWVRQAPGKGLEWVSVIYSGGSTYYADSVKGRFTISRDNSKNTLYLQMNSLRAEDTAVYYCARDSNAFDIWGQGTMVTVSS

SEQ ID NO: 13 - DNA, 339 bp, Artificial sequence
  Synthetic oligonucleotide
gaaattgtgctgactcagtctccactctccctgcccgtcacccctggagagccggcctccatctcctgcaggtctagtcagagcctcctgtatagtaatggatacaactatttggattggtacctgcagaagccagggaagtctccacaggtcctgatctatttgggttctaatcgggcctccggggtccccgacaggttcagtggcagtggatcaggcacagatttcacactgaaaatcagcagagtggaggctgaggatgttggggtttattactgcatgcaagctctacaaactccgatcaccttcggccaagggacacgactggagattaaacga

SEQ ID NO: 14 - protein, 113 aa, Artificial sequence
  Synthetic amino acid
EIVLTQSPLSLPVTPGEPASISCRSSQSLLYSNGYNYLDWYLQKPGKSPQVLIYLGSNRASGVPDRFSGSGSGTDFTLKISRVEAEDVGVYYCMQALQTPITFGQGTRLEIKR

SEQ ID NO: 15 - protein, 8 aa, Artificial sequence
  Synthetic amino acid
GFTVSSNY

SEQ ID NO: 16 - protein, 8 aa, Artificial sequence
  Synthetic amino acid
VIYSGGST

SEQ ID NO: 17 - protein, 9 aa, Artificial sequence
  Synthetic amino acid
ARDSNAFDI

SEQ ID NO: 18 - protein, 11 aa, Artificial sequence
  Synthetic amino acid
QSLLYSNGYNY

SEQ ID NO: 19 - protein, 3 aa, Artificial sequence
  Synthetic amino acid
LGS

SEQ ID NO: 20 - protein, 9 aa, Artificial sequence
  Synthetic amino acid
MQALQTPIT

SEQ ID NO: 21 - DNA, 366 bp, Artificial sequence
  Synthetic oligonucleotide
gaggtgcagctggtgcagtctgggggaggcttggtacagcctggggggtccctgagactctcctgtgcagcctctggattcacctttagcagctatgccatgagctgggtccgccaggctccagggaaggggctggagtgggtctcagctattagtggtagtggtggtagcacatactacgcagactccgtgaagggccgcttcaccatctccagagacaattccaagaacacgctgtctctgcaaatggacagcctgagacccgaggacacggccgtatattactgtgcgaaaagtcgagatagtgggaactaccttgatgcttttgatttctggggccaagggacaatggtcaccgtctcttca

SEQ ID NO: 22 - protein, 122 aa, Artificial sequence
  Synthetic amino acid
EVQLVQSGGGLVQPGGSLRLSCAASGFTFSSYAMSWVRQAPGKGLEWVSAISGSGGSTYYADSVKGRFTISRDNSKNTLSLQMDSLRPEDTAVYYCAKSRDSGNYLDAFDFWGQGTMVTVSS

SEQ ID NO: 23 - DNA, 324 bp, Artificial sequence
  Synthetic oligonucleotide
gacatccagttgacccagtctccttccaccctgtctgcatctgtaggagacagagtcaccatcacttgccgggccagtcagagtattagtagctggttggcctggtatcagcagaaagcagggaaagctcctaggctcctgatctatgatgcctccactttggaaagtggagtcccatcaaggttcagcggcactggatctgggacatatttcactctcaccatcagcagcctgcagcctgaagattttgcaacttattactgtcaacagtttaatagtttcccgctcactttcggcggagggaccaaggtggagatcaaacga

SEQ ID NO: 24 - protein, 108 aa, Artificial sequence
  Synthetic amino acid
DIQLTQSPSTLSASVGDRVTITCRASQSISSWLAWYQQKAGKAPRLLIYDASTLESGVPSRFSGTGSGTYFTLTISSLQPEDFATYYCQQFNSFPLTFGGGTKVEIKR

SEQ ID NO: 25 - protein, 8 aa, Artificial sequence
  Synthetic amino acid
GFTFSSYA

SEQ ID NO: 26 - protein, 8 aa, Artificial sequence
  Synthetic amino acid
ISGSGGST

SEQ ID NO: 27 - protein, 15 aa, Artificial sequence
  Synthetic amino acid
AKSRDSGNYLDAFDF

SEQ ID NO: 28 - protein, 6 aa, Artificial sequence
  Synthetic amino acid
QSISSW

SEQ ID NO: 29 - protein, 3 aa, Artificial sequence
  Synthetic amino acid
DAS

SEQ ID NO: 30 - protein, 9 aa, Artificial sequence
  Synthetic amino acid
QQFNSFPLT